European Patent Specification EP 3 574 918 B1, published October 15, 2025. Title: AGENT AND METHOD FOR TREATING OR PREVENTING RADIATION DAMAGE. Applicant: Kyowa Hakko Kirin Co., Ltd. The University of Tokyo. The sequence listing filed with the application follows.

SEQUENCE LISTING (17 sequences)

SEQ ID NO: 1 - protein, 5 aa, Artificial Sequence
  Amino acid sequence of  HCDR1 of Benralizumab
SYVIH

SEQ ID NO: 2 - protein, 17 aa, Artificial Sequence
  Amino acid sequence of  HCDR2 of Benralizumab
YINPYNDGTKYNERFKG

SEQ ID NO: 3 - protein, 12 aa, Artificial Sequence
  Amino acid sequence of  HCDR3 of Benralizumab
EGIRYYGLLGDY

SEQ ID NO: 4 - protein, 11 aa, Artificial Sequence
  Amino acid sequence of  LCDR1 of Benralizumab
GTSEDIINYLN

SEQ ID NO: 5 - protein, 7 aa, Artificial Sequence
  Amino acid sequence of  LCDR2 of Benralizumab
HTSRLQS

SEQ ID NO: 6 - protein, 9 aa, Artificial Sequence
  Amino acid sequence of  LCDR3 of Benralizumab
QQGYTLPYT

SEQ ID NO: 7 - protein, 121 aa, Artificial Sequence [sequence omitted]

SEQ ID NO: 8 - protein, 107 aa, Artificial Sequence [sequence omitted]

SEQ ID NO: 9 - protein, 451 aa, Artificial Sequence
  Amino acid sequence of heavy chain of Benralizumab
EVQLVQSGAEVKKPGASVKVSCKASGYTFTSYVIHWVRQRPGQGLAWMGYINPYNDGTKYNERFKGKVTITSDRSTSTVYMELSSLRSEDTAVYLCGREGIRYYGLLGDYWGQGTLVTVSSASTKGPSVFPLAPSSKSTSGGTAALGCLVKDYFPEPVTVSWNSGALTSGVHTFPAVLQSSGLYSLSSVVTVPSSSLGTQTYICNVNHKPSNTKVDKKVEPKSCDKTHTCPPCPAPELLGGPSVFLFPPKPKDTLMISRTPEVTCVVVDVSHEDPEVKFNWYVDGVEVHNAKTKPREEQYNSTYRVVSVLTVLHQDWLNGKEYKCKVSNKALPAPIEKTISKAKGQPREPQVYTLPPSRDELTKNQVSLTCLVKGFYPSDIAVEWESNGQPENNYKTTPPVLDSDGSFFLYSKLTVDKSRWQQGNVFSCSVMHEALHNHYTQKSLSLSPGK

SEQ ID NO: 10 - protein, 155 aa, Artificial Sequence
  Amino acid sequence of light chain of Benralizumab
DIQMTQSPSSLSASVGDRVTITCGTSEDIINYLNWYQQKPGKAPKLLIYHTSRLQSGVPSRFSGSGSGTDFTLTISSLQPEDFATYYCQQGYTLPYTFGQGTKVEIKRTVAAPSVFIFPPSDEQLKSGTASVVCLLNNFYPREAKVQWKVDNALQ

SEQ ID NO: 11 - DNA, 1248 bp, Rattus norvegicus
atggtgcctgtgttactaattcttgtgggagctttggcaacactgcaagctgacttacttaatcacaaaaagtttttacttctaccacctgtcaattttaccattaaagccactggattagctcaagttcttttacactgggacccaaatcctgaccaagagcaaaggcatgttgatctagagtatcacgtgaaaataaatgccccacaagaagacgaatatgataccagaaagactgaaagcaaatgtgtgaccccccttcatgaaggctttgcagctagcgtgaggaccattctgaagagcagccatacaactctggccagcagttgggtttctgctgaactcaaagctccaccaggatctcctggaacctcggttacgaatttaacttgtaccacacacactgttgtaagtagccacacccacttaaggccataccaagtgtcccttcgttgcacctggcttgttgggaaggatgcccctgaggacacacagtatttcctatactacaggtttggtgttttgactgaaaaatgccaagaatacagcagagatgcactgaacagaaatactgcatgctggtttcccaggacatttatcaacagcaaagggtttgagcagcttgctgtgcacattaatggctcaagcaagcgtgctgcaatcaagccctttgatcagctgttcagtccacttgccattgaccaagtgaatcctccaaggaatgtcacagtggaaattgaaagcaattctctctatatacagtgggagaaaccactttctgcctttccagatcattgctttaactatgagctgaaaatttacaacacaaaaaatggtcacattcagaaggaaaaactgatcgccaataagttcatctcaaaaattgatgatgtttctacatattccattcaagtgagagcagctgtgagctcaccttgcagaatgccaggaaggtggggcgagtggagtcaacctatttatgtgggaaaggaaaggaagtccttggtagaatggcatctcattgtgctcccaacagccgcctgcttcgtcttgttaatcttctcactcatctgcagagtgtgtcatctatggaccaggttgtttccaccggttccggccccaaagagtaacatcaaagatctccctgtggttactgaatatgagaaaccttcgaatgaaaccaaaattgaagttgtacattgtgtggaagaggttggatttgaagtcatgggaaattccacgttttga

SEQ ID NO: 12 - DNA, 411 bp, Rattus norvegicus
  CDS (1)..(411)
atggacatcaggctcagcttggttttccttgtccttttcataaaaggtgtccagtgtgaggtgcagctggtggagtctgatggaggcttagtacaacctggaaggtccctaaaactctcctgtgcagcctcaggattcactttcagtgacttttacatggcctgggtccgccaggctccaacgaaggggctggaatgggtcgcaaccattagttatgatggtagtagcgcttactatcgagactccgtgaagggccgattcactatctccagagataatgcaaaaagcaccctatacctgcaaatggacagtctgagctctgaggacacggccacttattactgtgcaagacatgacggttattacccctttgattactggggccaaggagtcatggtcacagtctcctca

SEQ ID NO: 13 - protein, 137 aa, Rattus norvegicus
MDIRLSLVFLVLFIKGVQCEVQLVESDGGLVQPGRSLKLSCAASGFTFSDFYMAWVRQAPTKGLEWVATISYDGSSAYYRDSVKGRFTISRDNAKSTLYLQMDSLSSEDTATYYCARHDGYYPFDYWGQGVMVTVSS

SEQ ID NO: 14 - protein, 117 aa, Rattus norvegicus
VQLVESDGGLVQPGRSLKLSCAASGFTFSDFYMAWVRQAPTKGLEWVATISYDGSSAYYRDSVKGRFTISRDNAKSTLYLQMDSLSSEDTATYYCARHDGYYPFDYWGQGVMVTVSS

SEQ ID NO: 15 - DNA, 378 bp, Rattus norvegicus
  CDS (1)..(378)
atgggtgtgcctactcatctcctgggtttgttgctgctctggattacacatgccatatgtgatatccggatgacacagtctccagcttccctgtctgcatctctgggagaaactgtcaacatcgaatgtctagcaagtgaggacatttacagtgatttagcatggtatcaacagaagccagggaaatctcctcagctcctgatctatgatgcaaatagcttgcaaaatggggtcccttcacggtttagtggcagtggatctggcacacagtattctctaaaaataaacagcctgcaatctgaagatgtcgcgacttatttctgtcaacaatataacaattattggacgttcggtggaggcaccaagctggaattgaaa

SEQ ID NO: 16 - protein, 126 aa, Rattus norvegicus
MGVPTHLLGLLLLWITHAICDIRMTQSPASLSASLGETVNIECLASEDIYSDLAWYQQKPGKSPQLLIYDANSLQNGVPSRFSGSGSGTQYSLKINSLQSEDVATYFCQQYNNYWTFGGGTKLELK

SEQ ID NO: 17 - protein, 106 aa, Rattus norvegicus
DIRMTQSPASLSASLGETVNIECLASEDIYSDLAWYQQKPGKSPQLLIYDANSLQNGVPSRFSGSGSGTQYSLKINSLQSEDVATYFCQQYNNYWTFGGGTKLELK